European Patent Specification EP 3 647 420 B1, published August 23, 2023. Title: A Probe and method for detecting a fusion gene and/or exon skipping. Applicant: The University of Tokyo. The sequence listing filed with the application follows.

SEQUENCE LISTING (12 sequences)

SEQ ID NO: 1 - DNA, 136 bp, Homo sapiens
aaatatgaaaagccaaaatttgtgcagtgtttagcattcttggggaatggagatgttcttactggagactcaggtggagtcatgcttatatggagcaaaactactgtagagcccacacctgggaaaggacctaaag

SEQ ID NO: 2 - DNA, 120 bp, Artificial
  probe
aatttgtgcagtgtttagcattcttggggaatggagatgttcttactggagactcaggtggagtcatgcttatatggagcaaaactactgtagagcccacacctgggaaaggacctaaag

SEQ ID NO: 3 - DNA, 120 bp, Artificial
  probe
aatatgaaaagccaaaatttgtgcagtgtttagcattcttggggaatggagatgttcttactggagactcaggtggagtcatgcttatatggagcaaaactactgtagagcccacacctg

SEQ ID NO: 4 - DNA, 120 bp, Artificial
  probe
agggaatttttgggaaatatgaaaagccaaaatttgtgcagtgtttagcattcttggggaatggagatgttcttactggagactcaggtggagtcatgcttatatggagcaaaactactg

SEQ ID NO: 5 - DNA, 120 bp, Artificial
  probe
cactaacaagaaaacagggaatttttgggaaatatgaaaagccaaaatttgtgcagtgtttagcattcttggggaatggagatgttcttactggagactcaggtggagtcatgcttatat

SEQ ID NO: 6 - DNA, 120 bp, Artificial
  probe
cctggagcggcaattcactaacaagaaaacagggaatttttgggaaatatgaaaagccaaaatttgtgcagtgtttagcattcttggggaatggagatgttcttactggagactcaggtg

SEQ ID NO: 7 - DNA, 187 bp, Homo sapiens
tgtaccgccggaagcaccaggagctgcaagccatgcagatggagctgcagagccctgagtacaagctgagcaagctccgcacctcgaccatcatgaccgactacaaccccaactactgctttgctggcaagacctcctccatcagtgacctgaaggaggtgccgcggaaaaacatcaccctcattcg

SEQ ID NO: 8 - DNA, 120 bp, Artificial
  probe
tgtaccgccggaagcaccaggagctgcaagccatgcagatggagctgcagagccctgagtacaagctgagcaagctccgcacctcgaccatcatgaccgactacaaccccaactactgct

SEQ ID NO: 9 - DNA, 120 bp, Artificial
  probe
caccaggagctgcaagccatgcagatggagctgcagagccctgagtacaagctgagcaagctccgcacctcgaccatcatgaccgactacaaccccaactactgctttgctggcaagacc

SEQ ID NO: 10 - DNA, 120 bp, Artificial
  probe
gccatgcagatggagctgcagagccctgagtacaagctgagcaagctccgcacctcgaccatcatgaccgactacaaccccaactactgctttgctggcaagacctcctccatcagtgac

SEQ ID NO: 11 - DNA, 120 bp, Artificial
  probe
ctgcagagccctgagtacaagctgagcaagctccgcacctcgaccatcatgaccgactacaaccccaactactgctttgctggcaagacctcctccatcagtgacctgaaggaggtgccg

SEQ ID NO: 12 - DNA, 120 bp, Artificial
  probe
gtacaagctgagcaagctccgcacctcgaccatcatgaccgactacaaccccaactactgctttgctggcaagacctcctccatcagtgacctgaaggaggtgccgcggaaaaacatcac